European Patent Specification EP 3 166 967 B1, published March 8, 2023. Title: SYNTHETIC SOMATOSTATIN RECEPTOR LIGANDS. Applicant: Tel HaShomer Medical Research Infrastructure and Services Ltd. Ramot at Tel Aviv University Ltd. KOSTENICH, Genady ORON-HERMAN, Mor ORENSTEIN, Arie SHEKHTER, Talia GAZIT, Ehud SALITRA, Yoseph BUZHANSKY, Ludmilla. The sequence listing filed with the application follows.

SEQUENCE LISTING (70 sequences)

SEQ ID NO: 1 - protein, 116 aa, HOMO_SAPIENS
  ref <308>: NP_001039
  ref <309>: 2015-03-15
  ref <313>: (1)..(116)
MLSCRLQCALAALSIVLALGCVTGAPSDPRLRQFLQKSLAAAAGKQELAKYFLAELLSEPNQTENDALEPEDLSQAAEQDEMRLELQRSANSNPAMAPRERKAGCKNFFWKTFTSC

SEQ ID NO: 2 - protein, 14 aa, HOMO_SAPIENS
AGCKNFFWKTFTSC

SEQ ID NO: 3 - protein, 28 aa, HOMO_SAPIENS
SANSNPAMAPRERKAGCKNFFWKTFTSC

SEQ ID NO: 4 - protein, 8 aa, ARTIFICIAL
  Synthetic peptide
  MOD_RES (1)..(1): D-naphthylalanine (D-Nal)
  DISULFID (2)..(7)
XCYWKVCT

SEQ ID NO: 5 - protein, 8 aa, ARTIFICIAL
  Synthetic peptide
  MOD_RES (1)..(1): D-phenylalanine
  DISULFID (2)..(7)
  MOD_RES (4)..(4): D-tryptophan
  MOD_RES (8)..(8): L-threoninol
XCFXKTCX

SEQ ID NO: 6 - protein, 9 aa, ARTIFICIAL
  Synthetic peptide
  MOD_RES (1)..(1): D-phenylalanine
  MISC_FEATURE (1)..(1): FITC-GABA covalently attached to D-Phe at position 1
  MISC_FEATURE (1)..(1): Optional FITC-GABA covalently attached to D-Phe at position 1
  DISULFID (2)..(9)
  MOD_RES (5)..(5): D-tryptophan
  MOD_RES (9)..(9): N-Thioethyl glycine
  ref <310>: US7,700,717
  ref <311>: 2004-09-24
  ref <312>: 2010-04-20
  ref <313>: (1)..(9)
XCFWXKTFX

SEQ ID NO: 7 - protein, 6 aa, ARTIFICIAL
  Synthetic peptide
  MISC_FEATURE (1)..(1): selected from the group consisting of Phe and Tyr
  MISC_FEATURE (1)..(4): at least one of: X at position 1 is Tyr,  X at position 2 is present or absent but if present is Phe, X at position 4 is other than Lys
  MISC_FEATURE (2)..(2): present or absent and if present is selected from the group consisting of Trp and Phe
  MOD_RES (3)..(3): D-tryptophan
  MISC_FEATURE (4)..(4): group consisting of amino acid residues having a side chain with at least one nitrogen atom
  MISC_FEATURE (6)..(6): "A" a chemical entity covalently attached to Phe
XXXXTF

SEQ ID NO: 8 - protein, 7 aa, ARTIFICIAL
  Synthetic peptide
  MISC_FEATURE (2)..(2): selected from the group consisting of Phe and Tyr
  MISC_FEATURE (2)..(5): at least one of: X at position 2 is Tyr,  X at position 3 is present or absent but if present is Phe, X at position 5 is other than Lys
  MISC_FEATURE (3)..(3): s present or absent and if present is selected from the group consisting of Trp and Phe
  MOD_RES (4)..(4): D-Tryptophan
  MISC_FEATURE (5)..(5): selected from the group consisting of amino acid residues having a side chain with at least one nitrogen atom
  MISC_FEATURE (7)..(7): "A" a chemical entity covalently attached to Phe
RXXXXTF

SEQ ID NO: 9 - protein, 8 aa, ARTIFICIAL
  Synthetic peptide
  MOD_RES (1)..(1): X is selected from HomoCysteine and D-Cysteine
  MOD_RES (1)..(1): X is selected from GlyS2, Cys, HomoCysteine and D-Cysteine
  MOD_RES (1)..(1): X is selected from Cysteine, HomoCysteine and D-Cysteine.
  MISC_FEATURE (2)..(2): X is present or absent but if present is Arg
  MISC_FEATURE (3)..(3): selected from the group consisting of Phe and Tyr
  MISC_FEATURE (4)..(4): X present or absent and if present is selected from the group consisting of Trp and Phe
  MOD_RES (5)..(5): D-tryptophan
  MISC_FEATURE (6)..(6): X is selected from the group consisting of amino acid residues having a side chain with at least one nitrogen atom
  MISC_FEATURE (8)..(8): "A" is a chemical entity covalently attached to Phe
XXXXXXTF

SEQ ID NO: 10 - protein, 9 aa, ARTIFICIAL
  Synthetic peptide
  MOD_RES (2)..(2): X selected from the group consisting of HomoCysteine and D-Cysteine
  MISC_FEATURE (3)..(3): X is present or absent but if present is Arg
  MISC_FEATURE (4)..(4): X is selected from the group consisting of Phe and Tyr
  MISC_FEATURE (5)..(5): X is present or absent and if present is selected from the group consisting of Trp and Phe
  MOD_RES (6)..(6): X is D-tryptophan
  MISC_FEATURE (7)..(7): X is selected from the group consisting of amino acid residues having a side chain with at least one nitrogen atom
  MISC_FEATURE (9)..(9): A chemical entity covalently bound to Phe
RXXXXXXTF

SEQ ID NO: 11 - protein, 10 aa, ARTIFICIAL
  Synthetic peptide
  MOD_RES (1)..(1): D-phenylalanine
  MISC_FEATURE (2)..(2): X is present or absent and if present is Arg
  MOD_RES (3)..(3): X is selected from the group consisting of HomoCysteine and D-Cysteine
  MISC_FEATURE (4)..(4): X is present or absent and if present is Arg
  MISC_FEATURE (5)..(5): X is selected from the group consisting of Phe and Tyr
  MISC_FEATURE (6)..(6): X is present or absent and if present is selected from the group consisting of Trp and Phe
  MOD_RES (7)..(7): D-tryptophan
  MISC_FEATURE (8)..(8): X is selected from the group consisting of amino acid residues having a side chain with at least one nitrogen atom
  BINDING (10)..(10): A chemical entity covalently bound to Phe
  MISC_FEATURE (10)..(10): A chemical entity covalently bound to Phe
XXXXXXXXTF

SEQ ID NO: 12 - protein, 9 aa, ARTIFICIAL
  Synthetic peptide
  MISC_FEATURE (1)..(1): Active agent Z or FITC-GABA covalently attached to D-Phe at position 1
  MOD_RES (1)..(1): D-Phenylalanine
  DISULFID (3)..(9)
  MOD_RES (5)..(5): D-Tryptophan
  MISC_FEATURE (9)..(9): N-Thioethyl glycine
XRCFXKTFX

SEQ ID NO: 13 - protein, 5 aa, ARTIFICIAL
  Synthetic peptide
  MOD_RES (2)..(2): D-tryptophan
  BINDING (5)..(5): "A" is a chemical entity covalently attached to Phe
FXKTF

SEQ ID NO: 14 - protein, 6 aa, ARTIFICIAL
  Synthetic peptide
  MOD_RES (3)..(3): D-tryptophan
  BINDING (6)..(6): "A" is a chemical entity covalently attached to Phe
CFXKTF

SEQ ID NO: 15 - protein, 7 aa, ARTIFICIAL
  Synthetic peptide
  MOD_RES (4)..(4): D-tryptophan
  BINDING (7)..(7): "A" is a chemical entity covalently attached to Phe
RCFXKTF

SEQ ID NO: 16 - protein, 8 aa, ARTIFICIAL
  Synthetic peptide
  MOD_RES (1)..(1): D-phenylalanine
  MOD_RES (5)..(5): D-tryptophan
  BINDING (8)..(8): "A" is a chemical entity covalently attached to Phe
XRCFXKTF

SEQ ID NO: 17 - protein, 9 aa, ARTIFICIAL
  Synthetic peptide
  MISC_FEATURE (1)..(1): Active agent Z or FITC-GABA covalently attached to D-Phe
  MOD_RES (1)..(1): D-Phenylalanine
  DISULFID (2)..(9)
  MOD_RES (5)..(5): D-Tryptophan
  MOD_RES (6)..(6): Ornithine
  MOD_RES (9)..(9): N-Thioethyl glycine
XCFWXXTFX

SEQ ID NO: 18 - protein, 6 aa, ARTIFICIAL
  Synthetic peptide
  MOD_RES (3)..(3): D-tryptophan
  MOD_RES (4)..(4): Ornithine
  BINDING (6)..(6): "A" is a chemical entity covalently attached to Phe
FWXXTF

SEQ ID NO: 19 - protein, 7 aa, ARTIFICIAL
  Synthetic peptide
  MOD_RES (4)..(4): D-Tryptophan
  MOD_RES (5)..(5): Ornithine
  BINDING (7)..(7): "A" is a chemical entity covalently attached to Phe
CFWXXTF

SEQ ID NO: 20 - protein, 8 aa, ARTIFICIAL
  Synthetic peptide
  MOD_RES (1)..(1): D-Phenylalanine
  MOD_RES (5)..(5): D-Tryptophan
  MOD_RES (6)..(6): Ornithine
  BINDING (8)..(8): "A" is a chemical entity covalently attached to Phe
XCFWXXTF

SEQ ID NO: 21 - protein, 9 aa, ARTIFICIAL
  Synthetic peptide
  MISC_FEATURE (1)..(1): Active agent Z or FITC-GABA covalently attached to D-Phe
  MOD_RES (1)..(1): D-Phenylalanine
  DISULFID (2)..(9)
  MOD_RES (5)..(5): D-Tryptophan
  MOD_RES (9)..(9): N-Thioethyl glycine
XCYWXKTFX

SEQ ID NO: 22 - protein, 6 aa, ARTIFICIAL
  Synthetic peptide
  MOD_RES (1)..(1): D-Tryptophan
  misc_feature (3)..(3): Xaa can be any naturally occurring amino acid
  BINDING (6)..(6): "A" is a chemical entity covalently attached to Phe
YWXKTF

SEQ ID NO: 23 - protein, 7 aa, ARTIFICIAL
  Synthetic peptide
  MOD_RES (4)..(4): D-Tryptophan
  BINDING (7)..(7): "A" is a chemical entity covalently attached to Phe
CYWXKTF

SEQ ID NO: 24 - protein, 8 aa, ARTIFICIAL
  Synthetic peptide
  MOD_RES (1)..(1): D-Phenylalanine
  MOD_RES (5)..(5): D-Tryptophan
  BINDING (8)..(8): "A" is a chemical entity covalently attached to Phe
XCYWXKTF

SEQ ID NO: 25 - protein, 9 aa, ARTIFICIAL
  Synthetic peptide
  MOD_RES (1)..(1): D-Phenylalanine
  MISC_FEATURE (1)..(1): Active agent Z or FITC-GABA covalently attached to DPhe
  MISC_FEATURE (1)..(1): FITC-GABA covalently attached to D-Phe at position 1
  DISULFID (3)..(9)
  MOD_RES (5)..(5): D-Tryptophan
  MOD_RES (6)..(6): Ornithine
  MOD_RES (9)..(9): N-Thioethyl glycine
XRCFXXTFX

SEQ ID NO: 26 - protein, 5 aa, ARTIFICIAL
  Synthetic peptide
  MOD_RES (2)..(2): D-Phenylalanine
  MOD_RES (3)..(3): Ornithine
  BINDING (5)..(5): "A" is a chemical entity covalently attached to Phe
FXXTF

SEQ ID NO: 27 - protein, 6 aa, ARTIFICIAL
  Synthetic peptide
  MOD_RES (3)..(3): D-Phenylalanine
  MOD_RES (4)..(4): Ornithine
  BINDING (6)..(6): "A" is a chemical entity covalently attached to Phe
CFXXTF

SEQ ID NO: 28 - protein, 7 aa, ARTIFICIAL
  Synthetic peptide
  MOD_RES (4)..(4): D-Phenylalanine
  MOD_RES (5)..(5): Ornithine
  BINDING (7)..(7): "A" is a chemical entity covalently attached to Phe
RCFXXTF

SEQ ID NO: 29 - protein, 8 aa, ARTIFICIAL
  Synthetic peptide
  MOD_RES (1)..(1): D-Phenylalanine
  MOD_RES (5)..(5): D-Tryptophan
  MOD_RES (6)..(6): Ornithine
  MOD_RES (8)..(8): "A" is a chemical entity covalently attached to Phe
XRCFXXTF

SEQ ID NO: 30 - protein, 9 aa, ARTIFICIAL
  Synthetic peptide
  MOD_RES (1)..(1): D-Phenylalanine
  MISC_FEATURE (1)..(1): Active agent Z or FITC-GABA covalently attached to DPhe
  MISC_FEATURE (1)..(1): FITC-GABA covalently attached to D-Phe at position 1
  DISULFID (3)..(9)
  MOD_RES (5)..(5): D-Tryptophan
  MOD_RES (9)..(9): N-Thioethyl glycine
XRCYXKTFX

SEQ ID NO: 31 - protein, 5 aa, ARTIFICIAL
  Synthetic peptide
  MOD_RES (2)..(2): D-Tryptophan
  BINDING (5)..(5): "A" is a chemical entity covalently attached to Phe
YXKTF

SEQ ID NO: 32 - protein, 6 aa, ARTIFICIAL
  Synthetic peptide
  MOD_RES (3)..(3): D-Phenylalanine
  BINDING (6)..(6): "A" is a chemical entity covalently attached to Phe
CYXKTF

SEQ ID NO: 33 - protein, 7 aa, ARTIFICIAL
  Synthetic peptide
  MOD_RES (4)..(4): D-Tryptophan
  BINDING (7)..(7): "A" is a chemical entity covalently attached to Phe
RCYXKTF

SEQ ID NO: 34 - protein, 8 aa, ARTIFICIAL
  Synthetic peptide
  MOD_RES (1)..(1): D-Phenylalanine
  MOD_RES (5)..(5): D-Tryptophan
  BINDING (8)..(8): "A" is a chemical entity covalently attached to Phe
XRCYXKTF

SEQ ID NO: 35 - protein, 8 aa, ARTIFICIAL
  Synthetic peptide
  MISC_FEATURE (1)..(1): Active agent Z or FITC-GABA covalently attached to DPhe
  MOD_RES (1)..(1): D-Phenylalanine
  DISULFID (2)..(8)
  MOD_RES (4)..(4): D-Tryptophan
  MOD_RES (5)..(5): Ornithine
  MOD_RES (8)..(8): N-Thioethyl glycine
XCYXXTFX

SEQ ID NO: 36 - protein, 5 aa, ARTIFICIAL
  Synthetic peptide
  MOD_RES (2)..(2): D-Tryptophan
  MOD_RES (3)..(3): Ornithine
  BINDING (5)..(5): "A" is a chemical entity covalently attached to Phe
YXXTF

SEQ ID NO: 37 - protein, 6 aa, ARTIFICIAL
  Synthetic peptide
  MOD_RES (3)..(3): D-Tryptophan
  MOD_RES (4)..(4): Ornithine
  BINDING (6)..(6): "A" is a chemical entity covalently attached to Phe
CYXXTF

SEQ ID NO: 38 - protein, 7 aa, ARTIFICIAL
  Synthetic peptide
  MOD_RES (1)..(1): D-Phenylalanine
  MOD_RES (4)..(4): D-Tryptophan
  MOD_RES (5)..(5): Ornithine
  BINDING (7)..(7): "A" is a chemical entity covalently attached to Phe
XCYXXTF

SEQ ID NO: 39 - protein, 10 aa, ARTIFICIAL
  Synthetic peptide
  MISC_FEATURE (1)..(1): Active agent Z or FITC-GABA covalently attached to DPhe
  MOD_RES (1)..(1): D-Phenylalanine
  DISULFID (2)..(10)
  MOD_RES (6)..(6): D-Tryptophan
  MOD_RES (10)..(10): N-Thioethyl glycine
XCRFFXKTFX

SEQ ID NO: 40 - protein, 5 aa, ARTIFICIAL
  Synthetic peptide
  MOD_RES (2)..(2): D-Tryptophan
  BINDING (5)..(5): "A" is a chemical entity covalently attached to Phe
FXKTF

SEQ ID NO: 41 - protein, 6 aa, ARTIFICIAL
  Synthetic peptide
  MOD_RES (3)..(3): D-Tryptophan
  BINDING (6)..(6): "A" is a chemical entity covalently attached to Phe
FFXKTF

SEQ ID NO: 42 - protein, 7 aa, ARTIFICIAL
  Synthetic peptide
  MOD_RES (3)..(3): D-Tryptophan
  misc_feature (4)..(4): Xaa can be any naturally occurring amino acid
  BINDING (7)..(7): "A" is a chemical entity covalently attached to Phe
RFFXKTF

SEQ ID NO: 43 - protein, 8 aa, ARTIFICIAL
  Synthetic peptide
  MOD_RES (5)..(5): D-Tryptophan
  BINDING (8)..(8): "A" is a chemical entity covalently attached to Phe
CRFFXKTF

SEQ ID NO: 44 - protein, 9 aa, ARTIFICIAL
  Synthetic peptide
  MOD_RES (1)..(1): D-Phenylalanine
  MOD_RES (6)..(6): D-Tryptophan
  BINDING (9)..(9): "A" is a chemical entity covalently attached to Phe
XCRFFXKTF

SEQ ID NO: 45 - protein, 8 aa, ARTIFICIAL
  Synthetic peptide
  MISC_FEATURE (1)..(1): Active agent Z or FITC-GABA covalently attached to  Cys at position 1
  DISULFID (1)..(8)
  MOD_RES (4)..(4): D-Tryptophan
  MOD_RES (8)..(8): N-Thioethyl glycine
CRFXKTFX

SEQ ID NO: 46 - protein, 9 aa, ARTIFICIAL
  Synthetic peptide
  MISC_FEATURE (1)..(1): Active agent Z or FITC-GABA covalently attached to DPhe at position 1
  MOD_RES (1)..(1): D-Phenylalanine
  DISULFID (2)..(9)
  MOD_RES (5)..(5): D-Tryptophan
  MOD_RES (9)..(9): N-Thioethyl glycine
XCRFXKTFX

SEQ ID NO: 47 - protein, 6 aa, ARTIFICIAL
  Synthetic peptide
  MOD_RES (3)..(3): D-Tryptophan
  BINDING (6)..(6): "A" is a chemical entity covalently attached to Phe
RFXKTF

SEQ ID NO: 48 - protein, 7 aa, ARTIFICIAL
  Synthetic peptide
  MOD_RES (4)..(4): D-Tryptophan
  BINDING (7)..(7): "A" is a chemical entity covalently attached to Phe
CRFXKTF

SEQ ID NO: 49 - protein, 8 aa, ARTIFICIAL
  Synthetic peptide
  MOD_RES (1)..(1): D-Phenylalanine
  MOD_RES (5)..(5): D-Tryptophan
  BINDING (8)..(8): "A" is a chemical entity covalently attached to Phe
XCRFXKTF

SEQ ID NO: 50 - protein, 9 aa, ARTIFICIAL
  Synthetic peptide
  MISC_FEATURE (1)..(1): Active agent Z or FITC-GABA covalently attached to D-Phe at position 1
  MOD_RES (1)..(1): D-Phenylalanine
  MOD_RES (2)..(2): HomoCysteine
  DISULFID (2)..(9)
  MOD_RES (5)..(5): D-Tryptophan
  MOD_RES (9)..(9): N-Thioethyl glycine
XXFWXKTFX

SEQ ID NO: 51 - protein, 8 aa, ARTIFICIAL
  Synthetic peptide
  MOD_RES (1)..(1): D-Phenylalanine
  MOD_RES (2)..(2): Homocysteine
  MOD_RES (5)..(5): D-Tryptophan
  BINDING (8)..(8): "A" is a chemical entity covalently attached to Phe
XXFWXKTF

SEQ ID NO: 52 - protein, 9 aa, ARTIFICIAL
  Synthetic peptide
  MISC_FEATURE (1)..(1): Active agent Z or FITC-GABA covalently attached to D-Phe at position 1
  MOD_RES (1)..(1): D-Phenylalanine
  MOD_RES (2)..(2): D-Cysteine
  DISULFID (2)..(9)
  MOD_RES (5)..(5): D-Tryptophan
  MOD_RES (9)..(9): N-Thioethyl glycine
XXFWXKTFX

SEQ ID NO: 53 - protein, 8 aa, ARTIFICIAL
  Synthetic peptide
  MOD_RES (1)..(1): D-Phenylalanine
  MOD_RES (2)..(2): D-Cysteine
  MOD_RES (5)..(5): D-Tryptophan
  BINDING (8)..(8): "A" is a chemical entity covalently attached to Phe
XXFWXKTF

SEQ ID NO: 54 - protein, 9 aa, ARTIFICIAL
  Synthetic peptide
  MISC_FEATURE (1)..(1): Active agent Z or FITC-GABA covalently attached to D-Phe at position 1
  MOD_RES (1)..(1): D-Phenylalanine
  DISULFID (2)..(9)
  MOD_RES (5)..(5): D-Tryptophan
  MOD_RES (6)..(6): 2-Aminoisobutyric acid
  MOD_RES (9)..(9): N-Thioethyl glycine
FCFWXXTFX

SEQ ID NO: 55 - protein, 6 aa, ARTIFICIAL
  Synthetic peptide
  MOD_RES (3)..(3): D-Phenylalanine
  MOD_RES (4)..(4): 2-Aminoisobutyric acid
  BINDING (6)..(6): "A" is a chemical entity covalently attached to Phe
FWXXTF

SEQ ID NO: 56 - protein, 7 aa, ARTIFICIAL
  Synthetic peptide
  MOD_RES (4)..(4): D-Phenylalanine
  MOD_RES (5)..(5): 2-Aminoisobutyric acid
  BINDING (7)..(7): "A" is a chemical entity covalently attached to Phe
CFWXXTF

SEQ ID NO: 57 - protein, 8 aa, ARTIFICIAL
  Synthetic peptide
  MOD_RES (1)..(1): D-Phenylalanine
  MOD_RES (5)..(5): D-Tryptophan
  MOD_RES (6)..(6): 2-Aminoisobutyric acid
  BINDING (8)..(8): "A" is a chemical entity covalently attached to Phe
XCFWXXTF

SEQ ID NO: 58 - protein, 9 aa, ARTIFICIAL
  Synthetic peptide
  MISC_FEATURE (1)..(1): Active agent Z or FITC-GABA covalently attached to D-Phe at position 1
  MOD_RES (1)..(1): D-Phenylalanine
  DISULFID (2)..(9)
  MOD_RES (5)..(5): D-Tryptophan
  MOD_RES (6)..(6): acetyllysine
  MOD_RES (9)..(9): N-Thioethyl glycine
XCFWXXTFX

SEQ ID NO: 59 - protein, 6 aa, ARTIFICIAL
  Synthetic peptide
  MOD_RES (3)..(3): D-Tryptophan
  MOD_RES (4)..(4): Acetyllysine
  BINDING (6)..(6): "A" is a chemical entity covalently attached to Phe
FWXXTF

SEQ ID NO: 60 - protein, 7 aa, ARTIFICIAL
  Synthetic peptide
  MOD_RES (4)..(4): D-Tryptophan
  MOD_RES (5)..(5): Acetyllysine
  BINDING (5)..(5): "A" is a chemical entity covalently attached to Phe
CFWXXTF

SEQ ID NO: 61 - protein, 8 aa, ARTIFICIAL
  Synthetic peptide
  MOD_RES (1)..(1): D-Phenylalanine
  MOD_RES (5)..(5): D-Tryptophan
  MOD_RES (6)..(6): acetyllysine
  BINDING (8)..(8): "A" is a chemical entity covalently attached to Phe
XCFWXXTF

SEQ ID NO: 62 - protein, 9 aa, ARTIFICIAL
  Synthetic peptide
  MISC_FEATURE (1)..(1): Active agent Z or FITC-GABA covalently attached to D-Phe at position 1
  MOD_RES (1)..(1): D-Phenylalanine
  DISULFID (2)..(9)
  MOD_RES (5)..(5): D-Tryptophan
  MOD_RES (9)..(9): N-Thioethyl glycine
XCFWXRTFX

SEQ ID NO: 63 - protein, 8 aa, ARTIFICIAL
  Synthetic peptide
  MOD_RES (1)..(1): D-Phenylalanine
  MOD_RES (5)..(5): D-Tryptophan
  BINDING (8)..(8): "A" is a chemical entity covalently attached to Phe
XCFWXRTF

SEQ ID NO: 64 - protein, 9 aa, ARTIFICIAL
  Synthetic peptide
  MISC_FEATURE (1)..(1): Active agent Z or FITC-GABA covalently attached to D-Phe at position 1
  MOD_RES (1)..(1): D-Phenylalanine
  DISULFID (2)..(9)
  MOD_RES (5)..(5): D-Tryptophan
  MOD_RES (6)..(6): HomoLysine
  MOD_RES (9)..(9): N-Thioethyl glycine
XCFWXXTFX

SEQ ID NO: 65 - protein, 6 aa, ARTIFICIAL
  Synthetic peptide
  MOD_RES (3)..(3): D-Tryptophan
  MOD_RES (4)..(4): HomoLysine
  BINDING (6)..(6): "A" is a chemical entity covalently attached to Phe
FWXXTF

SEQ ID NO: 66 - protein, 7 aa, ARTIFICIAL
  Synthetic peptide
  MOD_RES (4)..(4): D-Tryptophan
  MOD_RES (5)..(5): HomoLysine
  BINDING (7)..(7): "A" is a chemical entity covalently attached to Phe
CFWXXTF

SEQ ID NO: 67 - protein, 8 aa, ARTIFICIAL
  Synthetic peptide
  MOD_RES (1)..(1): D-Phenylalanine
  MOD_RES (5)..(5): D-Tryptophan
  MOD_RES (6)..(6): HomoLysine
  BINDING (8)..(8): "A" is a chemical entity covalently attached to Phe
XCFWXXTF

SEQ ID NO: 68 - protein, 9 aa, Artificial Sequence
  Synthetic peptide
  DISULFID (1)..(9)
  MISC_FEATURE (1)..(9): B' is any chemical entity covalently bonded to the terminal amino group of the N-terminal amino acid residue
  MOD_RES (2)..(8): Peptide is 6-9 amino acid residues, therefore three of the seven internal residues are optionally present or absent.
  MOD_RES (4)..(7): At least one of 4, 5, 6, 7 internal amino acids  includes a side chain functional group having a nitrogen atom (N) to which a nanoparticle active agent moiety is covalently attached (Q in Figure 13)
  MISC_FEATURE (9)..(9): B is any chemical entity covalently bonded to the terminal carbonyl group of the N-terminal amino acid residue
XXXXXXXXX

SEQ ID NO: 69 - protein, 8 aa, Artificial Sequence
  Synthetic peptide
  MOD_RES (1)..(1): N-Thioethyl glycine
  DISULFID (1)..(8)
  MOD_RES (4)..(4): D-tryptophan
  MOD_RES (8)..(8): N-Thioethyl glycine
  ref <310>: US 7,700,717
  ref <311>: 2004-09-24
  ref <312>: 2010-04-20
XFWXKTFX

SEQ ID NO: 70 - protein, 9 aa, Artificial Sequence
  Synthetic peptide
  MOD_RES (1)..(1 ): D-tryptophan
  MOD_RES (2)..(2): N-Thioethyl glycine
  DISULFID (2)..(9)
  MOD_RES (5)..(5): D-tryptophan
  MOD_RES (9)..(9): N-Thioethyl glycine
  ref <310>: US 7,700,717
  ref <311>: 2004-09-24
  ref <312>: 2010-04-20
XXFWXKTFX